European Patent Application EP 4 282 882 A2, published November 29, 2023. Title: BINDING DOMAINS DIRECTED AGAINST GPCR:G PROTEIN COMPLEXES AND USES DERIVED THEREOF. Applicant: VIB VZW. The sequence listing filed with the application follows.

SEQUENCE LISTING (73 sequences)

SEQ ID NO: 1 - protein, 138 aa, Lama glama
QVQLQESGGGLVQPGGSLRLSCAASGFTFSNYKMNWVRQAPGKGLEWVSDISQSGASISYTGSVKGRFTISRDNAKNTLYLQMNSLKPEDTAVYYCARCPAPFTRDCFDVTSTTYAYRGQGTQVTVSSHHHHHHEPEA

SEQ ID NO: 2 - protein, 138 aa, Lama glama
QVQLQESGGGLVQPGGSLRLSCAASGFTFSNYVMNWVRQAPGKGLEWVSDISNGGGTTSYASSVKGRFTISRDNAKNTLYLQMNGLKPADTAVYYCARCPAPFTNDCMDITSTTYAYRGQGTQVTVSSHHHHHHEPEA

SEQ ID NO: 3 - protein, 129 aa, Lama glama
QVQLQESGGGSVQAGGSLRLSCTVSGTIFSVTVMGWYRQAPGKQRELVAGFTNTRNTNYVDSVKGRFTISKDSAKNTMYLQMNSLKPEDTAVYYCNVRRWGGTNWNDYWGQGTQVTVSSHHHHHHEPEA

SEQ ID NO: 4 - protein, 129 aa, Lama glama
QVQLQESGGGFVQAGGSLRLSCAASGSIFSKNTMAWFRQAPGKERELVAASPTGGSTAYKDSVKGRFTISRDSAKNTVLLQMNVLKPEDTAVYYCHLRQNNRGSWFHYWGQGTQVTVSSHHHHHHEPEA

SEQ ID NO: 5 - protein, 129 aa, Lama glama
QVQLQESGGGLVQAGGSLRLSCAVSGTIFDITPMGWYRQTPGKQREVVADLTSRGTTNYADSVKGRFTISRDNAKKMLYLQMNSLKSDDTGVYYCNVKRWGGIGWNDYWGQGTQVTVSSHHHHHHEPEA

SEQ ID NO: 6 - protein, 129 aa, Lama glama
QVQLQESGGGLVQSGGSLRLSCVASGFRFSNFPMMWVRQAPGKGLEWVSLISIGGSTTNYADSVKGRFTISRDNAKNTLFLQMNSLKPEDTAVYYCAKYLGRLVPPTTEGQGTQVTVSSHHHHHHEPEA

SEQ ID NO: 7 - protein, 25 aa, Lama glama
QVQLQESGGGLVQPGGSLRLSCAAS

SEQ ID NO: 8 - protein, 25 aa, Lama glama
QVQLQESGGGLVQPGGSLRLSCAAS

SEQ ID NO: 9 - protein, 25 aa, Lama glama
QVQLQESGGGSVQAGGSLRLSCTVS

SEQ ID NO: 10 - protein, 25 aa, Lama glama
QVQLQESGGGFVQAGGSLRLSCAAS

SEQ ID NO: 11 - protein, 25 aa, Lama glama
QVQLQESGGGLVQAGGSLRLSCAVS

SEQ ID NO: 12 - protein, 25 aa, Lama glama
QVQLQESGGGLVQSGGSLRLSCVAS

SEQ ID NO: 13 - protein, 8 aa, Lama glama
GFTFSNYK

SEQ ID NO: 14 - protein, 8 aa, Lama glama
GFTFSNYV

SEQ ID NO: 15 - protein, 8 aa, Lama glama
GTIFSVTV

SEQ ID NO: 16 - protein, 8 aa, Lama glama
GSIFSKNT

SEQ ID NO: 17 - protein, 8 aa, Lama glama
GTIFDITP

SEQ ID NO: 18 - protein, 8 aa, Lama glama
GFRFSNFP

SEQ ID NO: 19 - protein, 17 aa, Lama glama
MNWVRQAPGKGLEWVSD

SEQ ID NO: 20 - protein, 17 aa, Lama glama
MNWVRQAPGKGLEWVSD

SEQ ID NO: 21 - protein, 17 aa, Lama glama
MGWYRQAPGKQRELVAG

SEQ ID NO: 22 - protein, 17 aa, Lama glama
MAWFRQAPGKERELVAA

SEQ ID NO: 23 - protein, 17 aa, Lama glama
MGWYRQTPGKQREVVAD

SEQ ID NO: 24 - protein, 17 aa, Lama glama
MMWVRQAPGKGLEWVSL

SEQ ID NO: 25 - protein, 8 aa, Lama glama
ISQSGASI

SEQ ID NO: 26 - protein, 8 aa, Lama glama
ISNGGGTT

SEQ ID NO: 27 - protein, 7 aa, Lama glama
FTNTRNT

SEQ ID NO: 28 - protein, 7 aa, Lama glama
SPTGGST

SEQ ID NO: 29 - protein, 7 aa, Lama glama
LTSRGTT

SEQ ID NO: 30 - protein, 8 aa, Lama glama
ISIGGSTT

SEQ ID NO: 31 - protein, 38 aa, Lama glama
SYTGSVKGRFTISRDNAKNTLYLQMNSLKPEDTAVYYC

SEQ ID NO: 32 - protein, 38 aa, Lama glama
SYASSVKGRFTISRDNAKNTLYLQMNGLKPADTAVYYC

SEQ ID NO: 33 - protein, 38 aa, Lama glama
NYVDSVKGRFTISKDSAKNTMYLQMNSLKPEDTAVYYC

SEQ ID NO: 34 - protein, 38 aa, Lama glama
AYKDSVKGRFTISRDSAKNTVLLQMNVLKPEDTAVYYC

SEQ ID NO: 35 - protein, 38 aa, Lama glama
NYADSVKGRFTISRDNAKKMLYLQMNSLKSDDTGVYYC

SEQ ID NO: 36 - protein, 38 aa, Lama glama
NYADSVKGRFTISRDNAKNTLFLQMNSLKPEDTAVYYC

SEQ ID NO: 37 - protein, 21 aa, Lama glama
ARCPAPFTRDCFDVTSTTYAY

SEQ ID NO: 38 - protein, 21 aa, Lama glama
ARCPAPFTNDCMDITSTTYAY

SEQ ID NO: 39 - protein, 13 aa, Lama glama
NVRRWGGTNWNDY

SEQ ID NO: 40 - protein, 13 aa, Lama glama
HLRQNNRGSWFHY

SEQ ID NO: 41 - protein, 13 aa, Lama glama
NVKRWGGIGWNDY

SEQ ID NO: 42 - protein, 12 aa, Lama glama
AKYLGRLVPPTT

SEQ ID NO: 43 - protein, 11 aa, Lama glama
RGQGTQVTVSS

SEQ ID NO: 44 - protein, 11 aa, Lama glama
RGQGTQVTVSS

SEQ ID NO: 45 - protein, 11 aa, Lama glama
WGQGTQVTVSS

SEQ ID NO: 46 - protein, 11 aa, Lama glama
WGQGTQVTVSS

SEQ ID NO: 47 - protein, 11 aa, Lama glama
WGQGTQVTVSS

SEQ ID NO: 48 - protein, 11 aa, Lama glama
EGQGTQVTVSS

SEQ ID NO: 49 - protein, 417 aa, Lama glama
CAGGTGCAGCTGCAGGAGTCTGGAGGAGGCTTGGTGCAGCCTGGGGGGTCTCTGAGACTCTCCTGTGCGGCCTCTGGATTCACCTTCAGCAATTATAAAATGAACTGGGTCCGCCAGGCTCCAGGAAAGGGGCTCGAGTGGGTCTCAGATATTTCTCAGAGTGGTGCTAGCATAAGTTACACAGGCTCCGTGAAGGGCCGATTCACCATCTCCAGAGACAACGCCAAGAACACGCTGTATCTACAAATGAACAGCCTGAAGCCTGAGGACACGGCCGTCTATTACTGTGCCAGATGTCCGGCCCCATTCACGAGAGATTGTTTTGACGTGACTAGTACCACGTATGCCTACAGGGGCCAGGGGACCCAGGTCACCGTCTCCTCACACCACCATCACCATCACGAACCTGAAGCCTAG

SEQ ID NO: 50 - protein, 417 aa, Lama glama
CAGGTGCAGCTGCAGGAGTCTGGAGGGGGCTTGGTGCAGCCTGGGGGGTCTCTGAGACTCTCCTGTGCAGCCTCTGGATTCACTTTCAGTAACTATGTCATGAACTGGGTCCGCCAGGCTCCAGGAAAGGGGCTCGAGTGGGTCTCAGATATTTCTAATGGCGGTGGTACCACAAGTTATGCAAGCTCCGTGAAGGGCCGATTCACCATCTCCAGAGACAACGCCAAGAACACGCTGTATCTGCAAATGAACGGCCTGAAGCCTGCGGACACGGCCGTCTATTACTGTGCAAGATGTCCGGCCCCATTCACGAACGATTGTATGGACATAACTAGTACCACGTATGCCTACAGGGGCCAGGGGACCCAGGTCACCGTCTCCTCACACCACCATCACCATCACGAACCTGAAGCCTAG

SEQ ID NO: 51 - protein, 390 aa, Lama glama
CAGGTGCAGCTGCAGGAGTCTGGAGGAGGCTCGGTGCAGGCTGGGGGGTCTCTGAGACTCTCCTGTACAGTCTCTGGAACCATCTTCAGTGTCACTGTCATGGGCTGGTACCGCCAGGCTCCAGGGAAGCAGCGCGAGTTGGTCGCAGGTTTTACTAATACTAGAAACACAAACTATGTAGACTCCGTGAAGGGCCGCTTCACCATCTCCAAAGACAGCGCCAAGAACACGATGTATCTACAAATGAACAGCCTGAAACCTGAGGACACAGCCGTCTATTACTGTAATGTACGTCGGTGGGGCGGTACGAATTGGAATGACTACTGGGGCCAGGGGACCCAGGTCACCGTCTCCTCACACCACCATCACCATCACGAACCTGAAGCCTAG

SEQ ID NO: 52 - protein, 390 aa, Lama glama
CAGGTGCAGCTGCAGGAGTCTGGAGGGGGCTTCGTGCAGGCTGGGGGGTCTCTGAGACTCTCCTGTGCAGCCTCTGGAAGCATCTTCAGTAAGAATACCATGGCCTGGTTCCGCCAGGCTCCAGGGAAGGAGCGAGAGTTGGTCGCAGCTAGTCCTACGGGTGGTAGCACAGCGTATAAAGACTCCGTGAAGGGCCGATTCACCATCTCCAGAGACAGCGCCAAGAACACGGTGTTGCTGCAAATGAACGTCCTGAAACCTGAGGATACTGCCGTCTATTACTGTCATCTACGTCAAAATAACCGTGGTTCTTGGTTCCACTACTGGGGCCAGGGGACCCAGGTCACCGTCTCCTCACACCACCATCACCATCACGAACCTGAAGCCTAG

SEQ ID NO: 53 - protein, 390 aa, Lama glama
CAGGTGCAGCTGCAGGAGTCTGGGGGAGGCTTGGTGCAGGCTGGGGGGTCGCTGAGACTCTCTTGTGCAGTCTCTGGTACGATCTTCGATATCACTCCCATGGGCTGGTACCGCCAGACTCCAGGGAAGCAGCGCGAAGTGGTCGCAGATCTTACTAGTCGCGGTACCACAAATTACGCAGACTCCGTGAAGGGCCGGTTCACCATCTCCAGAGACAACGCCAAGAAAATGTTGTATCTGCAAATGAACAGCCTGAAATCTGACGACACAGGCGTGTATTACTGTAACGTGAAACGGTGGGGAGGTATTGGCTGGAACGACTACTGGGGCCAGGGGACCCAGGTCACCGTCTCCTCACACCACCATCACCATCACGAACCTGAAGCCTAG

SEQ ID NO: 54 - protein, 390 aa, Lama glama
CAGGTGCAGCTGCAGGAGTCTGGAGGAGGCTTGGTGCAGTCTGGGGGGTCTCTGAGACTCTCCTGTGTAGCCTCTGGATTCAGATTCAGTAACTTTCCTATGATGTGGGTCCGCCAGGCCCCAGGAAAGGGGCTCGAGTGGGTCTCGCTGATTAGCATTGGTGGTAGTACCACGAATTATGCGGACTCCGTGAAGGGCCGATTCACCATCTCCAGAGACAACGCCAAGAACACGCTGTTTCTGCAAATGAACAGCCTGAAACCTGAGGACACGGCCGTGTATTACTGTGCAAAATATCTTGGTCGGCTGGTCCCACCGACTACTGAGGGCCAGGGGACCCAGGTCACCGTCTCCTCACACCACCATCACCATCACGAACCTGAAGCCTAG

SEQ ID NO: 55 - protein, 1095 aa, synthetic construct
  REGION 1..1095: note = Beta2AR construct
GGGCAACCCGGGAACGGCAGCGCCTTCTTGCTGGCACCCAATAGAAGCCATGCGCCGGACCACGACGTCACGCAGCAAAGGGACGAGGTGTGGGTGGTGGGCATGGGCATCGTCATGTCTCTCATCGTCCTGGCCATCGTGTTTGGCAATGTGCTGGTCATCACAGCCATTGCCAAGTTCGAGCGTCTGCAGACGGTCACCAACTACTTCATCACTTCACTGGCCTGTGCTGATCTGGTCATGGGCCTGGCAGTGGTGCCCTTTGGGGCCGCCCATATTCTTATGAAAATGTGGACTTTTGGCAACTTCTGGTGCGAGTTTTGGACTTCCATTGATGTGCTGTGCGTCACGGCCAGCATTGAGACCCTGTGCGTGATCGCAGTGGATCGCTACTTTGCCATTACTTCACCTTTCAAGTACCAGAGCCTGCTGACCAAGAATAAGGCCCGGGTGATCATTCTGATGGTGTGGATTGTGTCAGGCCTTACCTCCTTCTTGCCCATTCAGATGCACTGGTACCGGGCCACCCACCAGGAAGCCATCAACTGCTATGCCGAGGAGACCTGCTGTGACTTCTTCACGAACCAAGCCTATGCCATTGCCTCTTCCATCGTGTCCTTCTACGTTCCCCTGGTGATCATGGTCTTCGTCTACTCCAGGGTCTTTCAGGAGGCCAAAAGGCAGCTCCAGAAGATTGACAAATCTGAGGGCCGCTTCCATGTCCAGAACCTTAGCCAGGTGGAGCAGGATGGGCGGACGGGGCATGGACTCCGCAGATCTTCCAAGTTCTGCTTGAAGGAGCACAAAGCCCTCAAGACGTTAGGCATCATCATGGGCACTTTCACCCTCTGCTGGCTGCCCTTCTTCATCGTTAACATTGTGCATGTGATCCAGGATAACCTCATCCGTAAGGAAGTTTACATCCTCCTAAATTGGATAGGCTATGTCAATTCTGGTTTCAATCCCCTTATCTACTGCCGGAGCCCAGATTTCAGGATTGCCTTCCAGGAGCTTCTGTGCCTGCGCAGGTCTTCTTTGAAGGCCTATGGGAATGGCTACTCCAGCAACGGCAACACAGGGGAGCAGAGTGGATAA

SEQ ID NO: 56 - protein, 380 aa, Homo sapiens
MGCLGNSKTEDQRNEEKAQREANKKIEKQLQKDKQVYRATHRLLLLGAGESGKSTIVKQMRILHVNGFNGDSEKATKVQDIKNNLKEAIETIVAAMSNLVPPVELANPENQFRVDYILSVMNVPDFDFPPEFYEHAKALWEDEGVRACYERSNEYQLIDCAQYFLDKIDVIKQADYVPSDQDLLRCRVLTSGIFETKFQVDKVNFHMFDVGGQRDERRKWIQCFNDVTAIIFVVASSSYNMVIREDNQTNRLQEALNLFKSIWNNRWLRTISVILFLNKQDLLAEKVLAGKSKIEDYFPEFARYTTPEDATPEPGEDPRVTRAKYFIRDEFLRISTASGDGRHYCYPHFTCAVDTENIRRVFNDCRDIIQRMHLRQYELL

SEQ ID NO: 57 - protein, 354 aa, Homo sapiens
MGCTLSAEDKAAVERSKMIDRNLREDGEKAAREVKLLLLGAGESGKSTIVKQMKIIHEAGYSEEECKQYKAVVYSNTIQSIIAIIRAMGRLKIDFGDSARADDARQLFVLAGAAEEGFMTAELAGVIKRLWKDSGVQACFNRSREYQLNDSAAYYLNDLDRIAQPNYIPTQQDVLRTRVKTTGIVETHFTFKDLHFKMFDVGGQRSERKKWIHCFEGVTAIIFCVALSDYDLVLAEDEEMNRMHESMKLFDSICNNKWFTDTSIILFLNKKDLFEEKIKKSPLTICYPEYAGSNTYEEAAAYIQCQFEDLNKRKDTKEIYTHFTCATDTKNVQFVFDAVTDVIIKNNLKDCGLF

SEQ ID NO: 58 - protein, 350 aa, Homo sapiens
MGAGASAEEKHSRELEKKLKEDAEKDARTVKLLLLGAGESGKSTIVKQMKIIHQDGYSLEECLEFIAIIYGNTLQSILAIVRAMTTLNIQYGDSARQDDARKLMHMADTIEEGTMPKEMSDIIQRLWKDSGIQACFERASEYQLNDSAGYYLSDLERLVTPGYVPTEQDVLRSRVKTTGIIETQFSFKDLNFRMFDVGGQRSERKKWIHCFEGVTCIIFIAALSAYDMVLVEDDEVNRMHESLHLFNSICNHRYFATTSIVLFLNKKDVFFEKIKKAHLSICFPDYDGPNTYEDAGNYIKVQFLELNMRRDVKEIYSHMTCATDTQNVKFVFDAVTDIIIKENLKDCGLF

SEQ ID NO: 59 - protein, 394 aa, Bos taurus
MGCLGNSKTEDQRNEEKAQREANKKIEKQLQKDKQVYRATHRLLLLGAGESGKSTIVKQMRILHVNGFNGEGGEEDPQAARSNSDGEKATKVQDIKNNLKEAIETIVAAMSNLVPPVELANPENQFRVDYILSVMNVPDFDFPPEFYEHAKALWEDEGVRACYERSNEYQLIDCAQYFLDKIDVIKQDDYVPSDQDLLRCRVLTSGIFETKFQVDKVNFHMFDVGGQRDERRKWIQCFNDVTAIIFVVASSSYNMVIREDNQTNRLQEALNLFKSIWNNRWLRTISVILFLNKQDLLAEKVLAGKSKIEDYFPEFARYTTPEDATPEPGEDPRVTRAKYFIRDEFLRISTASGDGRHYCYPHFTCAVDTENIRRVFNDCRDIIQRMHLRQYELL

SEQ ID NO: 60 - protein, 394 aa, Rattus norvegicus
MGCLGNSKTEDQRNEEKAQREANKKIEKQLQKDKQVYRATHRLLLLGAGESGKSTIVKQMRILHVNGFNGEGGEEDPQAARSNSDGEKATKVQDIKNNLKEAIETIVAAMSNLVPPVELANPENQFRVDYILSVMNVPNFDFPPEFYEHAKALWEDEGVRACYERSNEYQLIDCAQYFLDKIDVIKQADYVPSDQDLLRCRVLTSGIFETKFQVDKVNFHMFDVGGQRDERRKWIQCFNDVTAIIFVVASSSYNMVIREDNQTNRLQEALNLFKSIWNNRWLRTISVILFLNKQDLLAEKVLAGKSKIEDYFPEFARYTTPEDATPEPGEDPRVTRAKYFIRDEFLRISTASGDGRHYCYPHFTCAVDTENIRRVFNDCRDIIQRMHLRQYELL

SEQ ID NO: 61 - protein, 394 aa, Mus musculus; identical to SEQ ID NO: 60

SEQ ID NO: 62 - protein, 340 aa, Bos taurus [sequence omitted]

SEQ ID NO: 63 - protein, 340 aa, Homo sapiens [sequence omitted]

SEQ ID NO: 64 - protein, 340 aa, Rattus norvegicus [sequence omitted]

SEQ ID NO: 65 - protein, 340 aa, Mus musculus [sequence omitted]

SEQ ID NO: 66 - protein, 71 aa, Bos taurus
MASNNTASIAQARKLVEQLKMEANIDRIKVSKAAADLMAYCEAHAKEDPLLTPVPASENPFREKKFFCAIL

SEQ ID NO: 67 - protein, 71 aa, Mus musculus; identical to SEQ ID NO: 66

SEQ ID NO: 68 - protein, 71 aa, Homo sapiens; identical to SEQ ID NO: 66

SEQ ID NO: 69 - protein, 514 aa, synthetic construct
  REGION 1..514: note = T4L-Beta2AR fusion construct
DYKDDDDAENLYFQGNIFEMLRIDEGLRLKIYKDTEGYYTIGIGHLLTKSPSLNAAKSELDKAIGRNTNGVITKDEAEKLFNQDVDAAVRGILRNAKLKPVYDSLDAVRRAALINMVFQMGETGVAGFTNSLRMLQQKRWDEAAVNLAKSRWYNQTPNRAKRVITTFRTGTWDAYAADEVWVVGMGIVMSLIVLAIVFGNVLVITAIAKFERLQTVTNYFITSLACADLVMGLAVVPFGAAHILTKTWTFGNFWCEFWTSIDVLCVTASIETLCVIAVDRYFAITSPFKYQSLLTKNKARVIILMVWIVSGLTSFLPIQMHWYRATHQEAINCYAEETCCDFFTNQAYAIASSIVSFYVPLVIMVFVYSRVFQEAKRQLQKIDKSEGRFHVQNLSQVEQDGRTGHGLRRSSKFCLKEHKALKTLGIIMGTFTLCWLPFFIVNIVHVIQDNLIRKEVYILLNWIGYVNSGFNPLIYCRSPDFRIAFQELLCLRRSSLKAYGNGYSSNGNTGEQSG

SEQ ID NO: 70 - protein, 8 aa, synthetic construct
  REGION 1..8: note = M1 Flag epitope
DYKDDDDA

SEQ ID NO: 71 - protein, 7 aa, synthetic construct
  REGION 1..7: note = TEV protease recognition sequence
ENLYFQG

SEQ ID NO: 72 - protein, 413 aa, Homo sapiens [sequence omitted]

SEQ ID NO: 73 - protein, 539 aa, synthetic construct [sequence omitted]